European Patent Specification EP 3 594 239 B1, published October 30, 2024. Title: METHODS FOR IMPROVING SAFETY OF BLOOD-BRAIN BARRIER TRANSPORT. Applicant: F. Hoffmann-La Roche AG. The sequence listing filed with the application follows.

SEQUENCE LISTING (15 sequences)

SEQ ID NO: 1 - protein, 108 aa, Artificial sequence
  sequence is synthesized
DIQMTQSPSSLSASVGDRVTITCRASQDVSTAVAWYQQKPGKAPKLLIYSASFLYSGVPSRFSGSGSGTDFTLTISSLQPEDFATYYCQQSYTTPPTFGQGTKVEIKR

SEQ ID NO: 2 - protein, 108 aa, Artificial sequence
  sequence is synthesized
DIQMTQSPSSLSASVGDRVTITCRASQDVSTAVAWYQQKPGKAPKLLIYSASFLYSGVPSRFSGSGSGTDFTLTISSLQPEDFATYYCQQFPTYLPTFGQGTKVEIKR

SEQ ID NO: 3 - protein, 108 aa, Artificial sequence
  sequence is synthesized
DIQMTQSPSSLSASVGDRVTITCRASQDVSTAVAWYQQKPGKAPKLLIYSASFLYSGVPSRFSGSGSGTDFTLTISSLQPEDFATYYCQQGYNDPPTFGQGTKVEIKR

SEQ ID NO: 4 - protein, 108 aa, Artificial sequence
  sequence is synthesized
DIQMTQSPSSLSASVGDRVTITCRASQDVSTAVAWYQQKPGKAPKLLIYSASFLYSGVPSRFSGSGSGTDFTLTISSLQPEDFATYYCQQSSTDPTTFGQGTKVEIKR

SEQ ID NO: 5 - protein, 108 aa, Artificial sequence
  sequence is synthesized
DIQMTQSPSSLSASVGDRVTITCRASQVVANSLAWYQQKPGKAPKLLIYLASFLYSGVPSRFSGSGSGTDFTLTISSLQPEDFATYYCQQDATSPPTFGQGTKVEIKR

SEQ ID NO: 6 - protein, 108 aa, Artificial sequence
  sequence is synthesized
DIQMTQSPSSLSASVGDRVTITCRASQDVSTAVAWYQQKPGKAPKLLIYSASFLYSGVPSRFSGSGSGTDFTLTISSLQPEDFATYYCQQYATDPPTFGQGTKVEIKR

SEQ ID NO: 7 - protein, 119 aa, Artificial sequence
  sequence is synthesized
EVQLVESGGGLVQPGGSLRLSCAASGFTFSGYAIHWVRQAPGKGLEWVGWISPAGGSTDYADSVKGRFTISADTSKNTAYLQMNSLRAEDTAVYYCARGPFSPWVMDYWGQGTLVTVSS

SEQ ID NO: 8 - protein, 119 aa, Artificial sequence
  sequence is synthesized
EVQLVESGGGLVQPGGSLRLSCAASGFTFLGYGIHWVRQAPGKGLEWVGWISPAGGSTDYADSVKGRFTISADTSKNTAYLQMNSLRAEDTAVYYCARGPFSPWVMDYWGQGTLVTVSS

SEQ ID NO: 9 - protein, 108 aa, Artificial sequence
  sequence is synthesized
DIQMTQSPSSLSASVGDRVTITCRASQSVSSAVAWYQQKPGKAPKLLIYSASSLYSGVPSRFSGSGSGTDFTLTISSLQPEDFATYYCQQYSYSPFTFGQGTKVEIKR

SEQ ID NO: 10 - protein, 108 aa, Artificial sequence
  sequence is synthesized
DIQMTQSPSSLSASVGDRVTITCRASQSVSSAVAWYQQKPGKAPKLLISWASWLYSGVPSRFSGSGSGTDFTLTISSLQPEDFATYYCQQYSYSPFTFGQGTKVEIKR

SEQ ID NO: 11 - protein, 108 aa, Artificial sequence
  sequence is synthesized
DIQMTQSPSSLSASVGDRVTITCRASQSVSSAVAWYQQKPGKAPKLLIWYASWLYSGVPSRFSGSGSGTDFTLTISSLQPEDFATYYCQQYSYSPFTFGQGTKVEIKR

SEQ ID NO: 12 - protein, 108 aa, Artificial sequence
  sequence is synthesized
DIQMTQSPSSLSASVGDRVTITCRASQSVSSAVAWYQQKPGKAPKLLIWWASSLYSGVPSRFSGSGSGTDFTLTISSLQPEDFATYYCQQYSYSPFTFGQGTKVEIKR

SEQ ID NO: 13 - protein, 126 aa, Artificial sequence
  sequence is synthesized
EVQLVESGGGLVQPGGSLRLSCAASGFNFYYSSIHWVRQAPGKGLEWVASISPYSGYTSYADSVKGRFTISADTSKNTAYLQMNSLRAEDTAVYYCARQPTHYYYYAKGYKAMDYWGQGTLVTVSS

SEQ ID NO: 14 - protein, 438 aa, Artificial sequence
  sequence is synthesized
EVQLVESGGGLVQPGGSLRLSCAASGFTFSSYGMSWVRQAPGKGLELVASINSNGGSTYYPDSVKGRFTISRDNAKNSLYLQMNSLRAEDTAVYYCASGDYWGQGTTVTVSSASTKGPSVFPLAPCSRSTSESTAALGCLVKDYFPEPVTVSWNSGALTSGVHTFPAVLQSSGLYSLSSVVTVPSSSLGTKTYTCNVDHKPSNTKVDKRVESKYGPPCPPCPAPEFLGGPSVFLFPPKPKDTLMISRTPEVTCVVVDVSQEDPEVQFNWYVDGVEVHNAKTKPREEQFNSTYRVVSVLTVLHQDWLNGKEYKCKVSNKGLPSSIEKTISKAKGQPREPQVYTLPPSQEEMTKNQVSLTCLVKGFYPSDIAVEWESNGQPENNYKTTPPVLDSDGSFFLYSRLTVDKSRWQEGNVFSCSVMHEALHNHYTQKSLSLSLG

SEQ ID NO: 15 - protein, 219 aa, Artificial sequence
  sequence is synthesized
DIVMTQSPLSLPVTPGEPASISCRSSQSLVYSNGDTYLHWYLQKPGQSPQLLIYKVSNRFSGVPDRFSGSGSGTDFTLKISRVEAEDVGVYYCSQSTHVPWTFGQGTKVEIKRTVAAPSVFIFPPSDEQLKSGTASVVCLLNNFYPREAKVQWKVDNALQSGNSQESVTEQDSKDSTYSLSSTLTLSKADYEKHKVYACEVTHQGLSSPVTKSFNRGEC